European Patent Specification EP 4 263 861 B1, published April 8, 2026. Title: COLORIMERIC METHOD FOR DETECTION OF AMPLIFIED GENETIC MATERIAL AND USES THEREOF. Applicant: UNIVERSIDADE NOVA DE LISBOA. The sequence listing filed with the application follows.

SEQUENCE LISTING (31 sequences)

SEQ ID NO: 1 - DNA, 42 bp, Artificial Sequence
  PCR primers gene N and in vitro RNA synthesis
taatacgactcactataggatgtctgataatggaccccaaaa

SEQ ID NO: 2 - DNA, 21 bp, Artificial Sequence
  PCR primer gene N
ttaggcctgagttgagtcagc

SEQ ID NO: 3 - DNA, 20 bp, Artificial Sequence
  PCR Primer PRS416 Fwd
gttttcccagtcacgacgtt

SEQ ID NO: 4 - DNA, 20 bp, Artificial Sequence
  PCR Primer PRS416 Rev
ttatgcttccggctcctatg

SEQ ID NO: 5 - DNA, 19 bp, SARS coronavirus 2
  RT-LAMP Primer GeneN-A-F3
tggctactaccgaagagct

SEQ ID NO: 6 - DNA, 20 bp, SARS coronavirus 2
  RT-LAMP Primer GeneN-A-B3
tgcagcattgttagcaggat

SEQ ID NO: 7 - DNA, 41 bp, SARS coronavirus 2
  RT-LAMP Primer GeneN-A-FIP
tctggcccagttcctaggtagtccagacgaattcgtggtgg

SEQ ID NO: 8 - DNA, 40 bp, SARS coronavirus 2
  RT-LAMP Primer GeneN-A-BIP
agacggcatcatatgggttgcacgggtgccaatgtgatct

SEQ ID NO: 9 - DNA, 25 bp, SARS coronavirus 2
  RT-LAMP Primer GeneN-A-LF
ggactgagatctttcattttaccgt

SEQ ID NO: 10 - DNA, 21 bp, SARS coronavirus 2
  RT-LAMP Primer GeneN-A-LB
actgagggagccttgaataca

SEQ ID NO: 11 - DNA, 17 bp, Candida albicans
  LAMP Primer Ca-F3
tctggtatccggagggc

SEQ ID NO: 12 - DNA, 20 bp, Candida albicans
  LAMP Primer Ca-B3
agtcctacctgatttgaggt

SEQ ID NO: 13 - DNA, 41 bp, Candida albicans
ctaccgtctttcaagcaaacccatgagcgtcgtttctccct

SEQ ID NO: 14 - DNA, 17 bp, Homo sapiens
  LAMP Primer RNaseP POP7 F3
ttgatgagctggagcca

SEQ ID NO: 15 - DNA, 18 bp, Homo sapiens
  LAMP Primer RNaseP POP7 B3
caccctcaatgcagagtc

SEQ ID NO: 16 - DNA, 20 bp, Homo sapiens
  LAMP Primer RNaseP POP7 LF
atgtggatggctgagttgtt

SEQ ID NO: 17 - DNA, 20 bp, Homo sapiens
  LAMP Primer RNaseP POP7 LB
catgctgagtactggacctc

SEQ ID NO: 18 - DNA, 41 bp, Homo sapiens
  LAMP Primer RNaseP POP7 FIP
gtgtgaccctgaagactcggttttagccactgactcggatc

SEQ ID NO: 19 - DNA, 45 bp, Homo sapiens
  LAMP Primer RNaseP POP7 BIP
cctccgtgatatggctcttcgtttttttcttacatggctctggtc

SEQ ID NO: 20 - DNA, 39 bp, Oryza sativa
  LAMP Primer Os-FIP
aacactccaggcctcaccgtggccgacctcattattccg

SEQ ID NO: 21 - DNA, 38 bp, Oryza sativa
  LAMP Primer Os-BIP
gttccggtccatcgatggctgcagcctctggagtgcta

SEQ ID NO: 22 - DNA, 20 bp, Oryza sativa
  LAMP Primer Os-F3
gacctcctcctagacctcaa

SEQ ID NO: 23 - DNA, 19 bp, Oryza sativa
  LAMP Primer Os-B3
tgacaaggcctgatcttgc

SEQ ID NO: 24 - DNA, 19 bp, Oryza sativa
  LAMP Primer Os-LF
ggaacatcaccggagacgg

SEQ ID NO: 25 - DNA, 17 bp, Oryza sativa
  LAMP Primer Os-LB
gcggcctgctttggctt

SEQ ID NO: 26 - DNA, 23 bp, [Clostridium] difficile
  LAMP Primer HK101-F3
gtatcaactgcattagatgaaac

SEQ ID NO: 27 - DNA, 22 bp, [Clostridium] difficile
  LAMP Primer HK101-B3
ccaaagatgaagtaatgattgc

SEQ ID NO: 28 - DNA, 48 bp, [Clostridium] difficile
  LAMP Primer HK101-FIP
ctgcacctaaacttacaccatctatcttcctacattatctgaaggatt

SEQ ID NO: 29 - DNA, 44 bp, [Clostridium] difficile
  LAMP Primer HK101-BIP
gagctaagtgaaacgagtgacccgctgttgttaaatttactgcc

SEQ ID NO: 30 - DNA, 18 bp, [Clostridium] difficile
  LAMP Primer HK101-FL
aatagttgcaattatagg

SEQ ID NO: 31 - DNA, 26 bp, [Clostridium] difficile
  LAMP Primer HK101-BL
agacaagaaatagaagctaagatagg